European Patent Application EP 4 663 659 A1, published December 17, 2025. Title: MUC-1 CONDITIONAL CD40 AGONISTS. Applicant: Merck Patent GmbH. The sequence listing filed with the application follows.

SEQUENCE LISTING (23 sequences)

SEQ ID NO: 1 - protein, 8 aa, synthetic construct
GYSFTGHY

SEQ ID NO: 2 - protein, 8 aa, synthetic construct
IDPVTGGT

SEQ ID NO: 3 - protein, 13 aa, synthetic construct
AREVTGDRGQFDK

SEQ ID NO: 4 - protein, 120 aa, synthetic construct
EVQLVQSGAEVKKPGASVKVSCKASGYSFTGHYMHWVRQAPGQGLEWMGWIDPVTGGTKYAQKFQGWVTMTRDTSISTAYMELSRLRSDDTAVYYCAREVTGDRGQFDKWGQGTLVTVSS

SEQ ID NO: 5 - protein, 449 aa, synthetic construct
EVQLVQSGAEVKKPGASVKVSCKASGYSFTGHYMHWVRQAPGQGLEWMGWIDPVTGGTKYAQKFQGWVTMTRDTSISTAYMELSRLRSDDTAVYYCAREVTGDRGQFDKWGQGTLVTVSSASTKGPSVFPLAPSSKSTSGGTAALGCLVKDYFPEPVTVSWNSGALTSGVHTFPAVLQSSGLYSLSSVVTVPSSSLGTQTYICNVNHKPSNTKVDKRVEPKSCDKTHTCPPCPAPEAAGGPSVFLFPPKPKDTLMISRTPEVTCVVVDVSHEDPEVKFNWYVDGVEVHNAKTKPREEQYNSTYRVVSVLTVLHQDWLNGKEYKCKVSNKALPAPIEKTISKAKGQPREPQVYTLPPSREEMTKNQVSLTCLVKGFYPSDIAVEWESNGQPENNYKTTPPVLDSDGSFFLYSKLTVDKSRWQQGNVFSCSVMHEALHNHYTQKSLSLSPG

SEQ ID NO: 6 - protein, 6 aa, synthetic construct
NIGSKS

SEQ ID NO: 7 - skipped

SEQ ID NO: 8 - protein, 10 aa, synthetic construct
QVWDSSSDWV

SEQ ID NO: 9 - protein, 107 aa, synthetic construct
SYVLTQPPSVSVAPGKTARITCGGNNIGSKSVHWYQQKPGQAPVLVIYYGSNRPSGIPERFSGSNSGNTATLTISRVEAGDEADYYCQVWDSSSDWVFGGGTKLTVL

SEQ ID NO: 10 - protein, 213 aa, synthetic construct
SYVLTQPPSVSVAPGKTARITCGGNNIGSKSVHWYQQKPGQAPVLVIYYGSNRPSGIPERFSGSNSGNTATLTISRVEAGDEADYYCQVWDSSSDWVFGGGTKLTVLGQPKAAPSVTLFPPSSEELQANKATLVCLISDFYPGAVTVAWKADSSPVKAGVETTTPSKQSNNKYAASSYLSLTPEQWKSHKSYSCQVTHEGSTVEKTVAPTECS

SEQ ID NO: 11 - protein, 15 aa, synthetic construct
GSGGGSGGSGGGGSG

SEQ ID NO: 12 - protein, 8 aa, synthetic construct
GFTFSSAT

SEQ ID NO: 13 - protein, 8 aa, synthetic construct
ISSVGGGT

SEQ ID NO: 14 - protein, 14 aa, synthetic construct
VTMRSIRNPDFGSR

SEQ ID NO: 15 - protein, 121 aa, synthetic construct
EVQLVESGGGVVQPGGSLRLSCAASGFTFSSATMGWFRQAPGKGLEWVAYISSVGGGTDYADSVKGRFTISRDNAKNTLYLQMNSLRAEDTAVYYCVTMRSIRNPDFGSRGQGTLVTVSSA

SEQ ID NO: 16 - protein, 585 aa, synthetic construct
EVQLVQSGAEVKKPGASVKVSCKASGYSFTGHYMHWVRQAPGQGLEWMGWIDPVTGGTKYAQKFQGWVTMTRDTSISTAYMELSRLRSDDTAVYYCAREVTGDRGQFDKWGQGTLVTVSSASTKGPSVFPLAPSSKSTSGGTAALGCLVKDYFPEPVTVSWNSGALTSGVHTFPAVLQSSGLYSLSSVVTVPSSSLGTQTYICNVNHKPSNTKVDKRVEPKSCDKTHTCPPCPAPEAAGGPSVFLFPPKPKDTLMISRTPEVTCVVVDVSHEDPEVKFNWYVDGVEVHNAKTKPREEQYNSTYRVVSVLTVLHQDWLNGKEYKCKVSNKALPAPIEKTISKAKGQPREPQVYTLPPSREEMTKNQVSLTCLVKGFYPSDIAVEWESNGQPENNYKTTPPVLDSDGSFFLYSKLTVDKSRWQQGNVFSCSVMHEALHNHYTQKSLSLSPGGSGGGSGGSGGGGSGEVQLVESGGGVVQPGGSLRLSCAASGFTFSSATMGWFRQAPGKGLEWVAYISSVGGGTDYADSVKGRFTISRDNAKNTLYLQMNSLRAEDTAVYYCVTMRSIRNPDFGSRGQGTLVTVSSA

SEQ ID NO: 17 - DNA, 1821 bp, synthetic construct
  source 1..1821: mol_type = other DNA
atggaaacagacaccctgctgctgtgggtgctgctgctgtgggtgcccggctccacaggcgaggtgcagctggtgcagtctggggccgaggtgaagaaaccaggcgccagcgtgaaggtgtcctgcaaggccagcggctacagcttcaccggccactacatgcactgggtgcgccaggctccaggccagggactggaatggatgggctggatcgaccctgtgaccggcggcaccaaatacgcccagaagttccagggctgggtcaccatgacccgggacaccagcatcagcaccgcctacatggaactgagccggctgagaagcgacgacaccgccgtgtactactgcgccagagaagtgacaggcgaccggggccagttcgataagtggggccagggcacactcgtgaccgtgagcagcgcctccaccaagggcccatcggtcttccccctggcaccctcctccaagagcacctctgggggcacagcggccctgggctgcctggtcaaggactacttccccgaaccggtgacggtgtcgtggaactcaggcgccctgaccagcggcgtgcacaccttcccggctgtcctacagtcctcaggactctactccctcagcagcgtggtgaccgtgccctccagcagcttgggcacccagacctacatctgcaacgtgaatcacaagcccagcaacaccaaggtggacaagagagttgaacccaagagctgcgacaagacccacacctgtcctccatgtcctgctcctgaagctgccgggggcccttccgtgtttctgttccctccaaagcctaaggacaccctgatgatcagcagaacccctgaagtgacctgcgtggtggtggatgtgtctcacgaggaccccgaagtgaagttcaattggtacgtggacggcgtggaagttcacaacgcaaagactaaacctcgagaagagcagtataattctacatatcgtgtcgtgtccgttctcaccgtgctccaccaggattggttgaatggcaaagagtataagtgcaaggtgtccaacaaagcacttccagcacccatcgaaaagaccatttctaaggccaaggggcaaccccgagaacctcaagtgtatactctgcccccttctcgcgaagagatgactaaaaaccaggtcagtcttacttgcttggtcaaaggcttctaccctagcgacatcgccgtcgaatgggaaagcaatgggcaaccagaaaataactacaagacaaccccacctgtcctcgattcagacggcagtttttttctgtatagtaaactgacagtggacaaaagccgctggcagcagggtaacgtcttttcatgttcagttatgcatgaggcacttcacaatcattacacccaaaagagcctgtctctcagtccaggtggtagtggtggcgggtctggaggctcaggcgggggtggttcaggggaagtacagctcgtagaatcaggaggaggggtggtccaaccaggcggctcactgcgactgtcatgcgcagcttcaggattcacattcagctctgcaaccatgggctggtttaggcaagcccccggaaaggggctcgaatgggtcgcatacatttcatccgtaggggggggtactgattacgcagactcagtaaagggacgttttacaatatctcgcgacaatgcaaaaaatacactgtatcttcaaatgaactcactcagggctgaggataccgccgtatattactgtgtcacaatgcggtcaatacgtaacccagactttgggtcacgggggcaagggacactcgtgacagtttcatctgcataatga

SEQ ID NO: 18 - DNA, 705 bp, synthetic construct
  source 1..705: mol_type = other DNA
atgcgggctctcctggccaggctgctgctgtgcgtgctggtggtgagcgacagcaagggcagctacgtgctgactcagcctcctagcgtcagcgtggctcccggcaaaactgctaggatcacatgtggcggcaacaacatcggcagcaagagcgtgcactggtatcagcagaagcccggccaagccccagtgctcgtgatctactacggcagcaataggccttccggcatcccagagagattctccggcagcaactccggcaatactgccacactgacaatctctagggtggaggccggagacgaggctgactactattgccaagtgtgggacagcagctccgactgggtgttcggcggaggcactaagctgactgtgctgggacagcctaaggccgctcctagcgtgactctgttcccaccaagcagcgaggagctgcaagccaataaagccactctggtgtgtctgatcagcgatttctaccccggcgccgtgacagtcgcttggaaggctgattccagcccagtgaaggccggcgtggagactacaactccttccaagcagtccaacaacaagtacgccgccagctcctatctgtctctgactccagagcagtggaagagccacaagagctacagctgccaagtgactcacgagggctccactgtggagaagacagtggcccctacagagtgcagctgatag

SEQ ID NO: 19 - protein, 605 aa, synthetic construct
METDTLLLWVLLLWVPGSTGEVQLVQSGAEVKKPGASVKVSCKASGYSFTGHYMHWVRQAPGQGLEWMGWIDPVTGGTKYAQKFQGWVTMTRDTSISTAYMELSRLRSDDTAVYYCAREVTGDRGQFDKWGQGTLVTVSSASTKGPSVFPLAPSSKSTSGGTAALGCLVKDYFPEPVTVSWNSGALTSGVHTFPAVLQSSGLYSLSSVVTVPSSSLGTQTYICNVNHKPSNTKVDKRVEPKSCDKTHTCPPCPAPEAAGGPSVFLFPPKPKDTLMISRTPEVTCVVVDVSHEDPEVKFNWYVDGVEVHNAKTKPREEQYNSTYRVVSVLTVLHQDWLNGKEYKCKVSNKALPAPIEKTISKAKGQPREPQVYTLPPSREEMTKNQVSLTCLVKGFYPSDIAVEWESNGQPENNYKTTPPVLDSDGSFFLYSKLTVDKSRWQQGNVFSCSVMHEALHNHYTQKSLSLSPGGSGGGSGGSGGGGSGEVQLVESGGGVVQPGGSLRLSCAASGFTFSSATMGWFRQAPGKGLEWVAYISSVGGGTDYADSVKGRFTISRDNAKNTLYLQMNSLRAEDTAVYYCVTMRSIRNPDFGSRGQGTLVTVSSA

SEQ ID NO: 20 - protein, 233 aa, synthetic construct
MRALLARLLLCVLVVSDSKGSYVLTQPPSVSVAPGKTARITCGGNNIGSKSVHWYQQKPGQAPVLVIYYGSNRPSGIPERFSGSNSGNTATLTISRVEAGDEADYYCQVWDSSSDWVFGGGTKLTVLGQPKAAPSVTLFPPSSEELQANKATLVCLISDFYPGAVTVAWKADSSPVKAGVETTTPSKQSNNKYAASSYLSLTPEQWKSHKSYSCQVTHEGSTVEKTVAPTECS

SEQ ID NO: 21 - protein, 1255 aa, Homo sapiens
MTPGTQSPFFLLLLLTVLTVVTGSGHASSTPGGEKETSATQRSSVPSSTEKNAVSMTSSVLSSHSPGSGSSTTQGQDVTLAPATEPASGSAATWGQDVTSVPVTRPALGSTTPPAHDVTSAPDNKPAPGSTAPPAHGVTSAPDTRPAPGSTAPPAHGVTSAPDTRPAPGSTAPPAHGVTSAPDTRPAPGSTAPPAHGVTSAPDTRPAPGSTAPPAHGVTSAPDTRPAPGSTAPPAHGVTSAPDTRPAPGSTAPPAHGVTSAPDTRPAPGSTAPPAHGVTSAPDTRPAPGSTAPPAHGVTSAPDTRPAPGSTAPPAHGVTSAPDTRPAPGSTAPPAHGVTSAPDTRPAPGSTAPPAHGVTSAPDTRPAPGSTAPPAHGVTSAPDTRPAPGSTAPPAHGVTSAPDTRPAPGSTAPPAHGVTSAPDTRPAPGSTAPPAHGVTSAPDTRPAPGSTAPPAHGVTSAPDTRPAPGSTAPPAHGVTSAPDTRPAPGSTAPPAHGVTSAPDTRPAPGSTAPPAHGVTSAPDTRPAPGSTAPPAHGVTSAPDTRPAPGSTAPPAHGVTSAPDTRPAPGSTAPPAHGVTSAPDTRPAPGSTAPPAHGVTSAPDTRPAPGSTAPPAHGVTSAPDTRPAPGSTAPPAHGVTSAPDTRPAPGSTAPPAHGVTSAPDTRPAPGSTAPPAHGVTSAPDTRPAPGSTAPPAHGVTSAPDTRPAPGSTAPPAHGVTSAPDTRPAPGSTAPPAHGVTSAPDTRPAPGSTAPPAHGVTSAPDTRPAPGSTAPPAHGVTSAPDTRPAPGSTAPPAHGVTSAPDTRPAPGSTAPPAHGVTSAPDTRPAPGSTAPPAHGVTSAPDTRPAPGSTAPPAHGVTSAPDTRPAPGSTAPPAHGVTSAPDTRPAPGSTAPPAHGVTSAPDTRPAPGSTAPPAHGVTSAPDTRPAPGSTAPPAHGVTSAPDNRPALGSTAPPVHNVTSASGSASGSASTLVHNGTSARATTTPASKSTPFSIPSHHSDTPTTLASHSTKTDASSTHHSSVPPLTSSNHSTSPQLSTGVSFFFLSFHISNLQFNSSLEDPSTDYYQELQRDISEMFLQIYKQGGFLGLSNIKFRPGSVVVQLTLAFREGTINVHDVETQFNQYKTEAASRYNLTISDVSVSDVPFPFSAQSGAGVPGWGIALLVLVCVLVALAIVYLIALAVCQCRRKNYGQLDIFPARDTYHPMSEYPTYHTHGRYVPPSSTDRSPYEKVSAGNGGSSLSYTNPAVAATSANL

SEQ ID NO: 22 - protein, 277 aa, Homo sapiens
MVRLPLQCVLWGCLLTAVHPEPPTACREKQYLINSQCCSLCQPGQKLVSDCTEFTETECLPCGESEFLDTWNRETHCHQHKYCDPNLGLRVQQKGTSETDTICTCEEGWHCTSEACESCVLHRSCSPGFGVKQIATGVSDTICEPCPVGFFSNVSSAFEKCHPWTSCETKDLVVQQAGTNKTDVVCGPQDRLRALVVIPIIFGILFAILLVLVFIKKVAKKPTNKAPHPKQEPQEINFPDDLPGSNTAAPVQETLHGCQPVTQEDGKESRISVQERQ

SEQ ID NO: 23 - protein, 15 aa, synthetic construct
APDTRPAPGSTAPPA